European Patent Specification EP 4 416 205 B1, published December 10, 2025. Title: Zwitterionic functionalized poly(beta-aminoester) polymers and uses thereof. Applicant: INSTITUT QUIMIC DE SARRIA CETS FUNDACIO PRIVADA. The sequence listing filed with the application follows.

SEQUENCE LISTING (2 sequences)

SEQ ID NO: 1 - protein, 4 aa, synthetic construct
  REGION 1..4: note = peptide
CKKK

SEQ ID NO: 2 - protein, 4 aa, synthetic construct
  REGION 1..4: note = peptide
CHHH